European Patent Application EP 4 628 592 A1, published October 8, 2025. Title: 特定位置に酸素原子を有するアミノ酸を翻訳する工程を含む、ペプチドの製造方法. Applicant: 中外製薬株式会社. The sequence listing filed with the application follows.

SEQUENCE LISTING (37 sequences)

SEQ ID NO: 1 - RNA, 74 nt, synthetic construct
  source 1..74: mol_type = other RNA
gtccccttcgtctagaggcccaggacaccgcccttagacggcggtaacaggggttcgaatcccctaggggacgc

SEQ ID NO: 2 - RNA, 74 nt, synthetic construct
  source 1..74: mol_type = other RNA
gtccccttcgtctagaggcccaggacaccgccctctgacggcggtaacaggggttcgaatcccctaggggacgc

SEQ ID NO: 3 - RNA, 75 nt, synthetic construct
  source 1..75: mol_type = other RNA
ggcggggtggagcagcctggtagctcgtcgggctcataacccgaagatcgtcggttcaaatccggcccccgcaac

SEQ ID NO: 4 - DNA, 94 bp, synthetic construct
  source 1..94: mol_type = other DNA
gtaatacgactcactatagggttaactttaagaaggagatatacatatgatttttattggttttattattctacagattccgggttaagcttcg

SEQ ID NO: 5 - DNA, 94 bp, synthetic construct
  source 1..94: mol_type = other DNA
gtaatacgactcactatagggttaactttaagaaggagatatacatatgatttttattggttttattattcagctaattccgggttaagcttcg

SEQ ID NO: 6 - RNA, 76 nt, synthetic construct
  source 1..76: mol_type = other RNA
gggttaactttaagaaggagatatacatatgatttttattggttttattattctacagattccgggttaagcttcg

SEQ ID NO: 7 - RNA, 76 nt, synthetic construct
  source 1..76: mol_type = other RNA
gggttaactttaagaaggagatatacatatgatttttattggttttattattcagctaattccgggttaagcttcg

SEQ ID NO: 8 - protein, 13 aa, synthetic construct
  REGION 1..13: note = Peptide Compound
  SITE 1: note = MISC_FEATURE - Xaa = BdpF
  SITE 3: note = MISC_FEATURE - Xaa = MeF
  SITE 6: note = MISC_FEATURE - Xaa = MeF
  SITE 9: note = MISC_FEATURE - Xaa = nBuG
  SITE 10: note = MISC_FEATURE - Xaa = MeA
XIXIGXIIXXIPG

SEQ ID NO: 9 - protein, 13 aa, synthetic construct
  REGION 1..13: note = Peptide Compound
  SITE 1: note = MISC_FEATURE - Xaa = BdpF
  SITE 3: note = MISC_FEATURE - Xaa = MeF
  SITE 6: note = MISC_FEATURE - Xaa = MeF
  SITE 9: note = MISC_FEATURE - Xaa = MeOEtG
  SITE 10: note = MISC_FEATURE - Xaa = MeA
XIXIGXIIXXIPG

SEQ ID NO: 10 - protein, 13 aa, synthetic construct
  REGION 1..13: note = Peptide Compound
  SITE 1: note = MISC_FEATURE - Xaa = BdpF
  SITE 3: note = MISC_FEATURE - Xaa = MeF
  SITE 6: note = MISC_FEATURE - Xaa = MeF
  SITE 9: note = MISC_FEATURE - Xaa = MeOPrG
  SITE 10: note = MISC_FEATURE - Xaa = MeA
XIXIGXIIXXIPG

SEQ ID NO: 11 - protein, 13 aa, synthetic construct
  REGION 1..13: note = Peptide Compound
  SITE 1: note = MISC_FEATURE - Xaa = BdpF
  SITE 3: note = MISC_FEATURE - Xaa = MeF
  SITE 6: note = MISC_FEATURE - Xaa = MeF
  SITE 9: note = MISC_FEATURE - Xaa = PhPrG
  SITE 10: note = MISC_FEATURE - Xaa = MeA
XIXIGXIIXXIPG

SEQ ID NO: 12 - protein, 13 aa, synthetic construct
  REGION 1..13: note = Peptide Compound
  SITE 1: note = MISC_FEATURE - Xaa = BdpF
  SITE 3: note = MISC_FEATURE - Xaa = MeF
  SITE 6: note = MISC_FEATURE - Xaa = MeF
  SITE 9: note = MISC_FEATURE - Xaa = PhOEtG
  SITE 10: note = MISC_FEATURE - Xaa = MeA
XIXIGXIIXXIPG

SEQ ID NO: 13 - protein, 13 aa, synthetic construct
  REGION 1..13: note = Peptide Compound
  SITE 1: note = MISC_FEATURE - Xaa = BdpF
  SITE 3: note = MISC_FEATURE - Xaa = MeF
  SITE 6: note = MISC_FEATURE - Xaa = MeF
  SITE 9: note = MISC_FEATURE - Xaa = D-Nva
  SITE 10: note = MISC_FEATURE - Xaa = MeA
XIXIGXIIXXIPG

SEQ ID NO: 14 - protein, 13 aa, synthetic construct
  REGION 1..13: note = Peptide Compound
  SITE 1: note = MISC_FEATURE - Xaa = BdpF
  SITE 3: note = MISC_FEATURE - Xaa = MeF
  SITE 6: note = MISC_FEATURE - Xaa = MeF
  SITE 9: note = MISC_FEATURE - Xaa = D-Ser(Me)
  SITE 10: note = MISC_FEATURE - Xaa = MeA
XIXIGXIIXXIPG

SEQ ID NO: 15 - protein, 13 aa, synthetic construct
  REGION 1..13: note = Peptide Compound
  SITE 1: note = MISC_FEATURE - Xaa = BdpF
  SITE 3: note = MISC_FEATURE - Xaa = MeF
  SITE 6: note = MISC_FEATURE - Xaa = MeF
  SITE 9: note = MISC_FEATURE - Xaa = D-Hph
  SITE 10: note = MISC_FEATURE - Xaa = MeA
XIXIGXIIXXIPG

SEQ ID NO: 16 - protein, 13 aa, synthetic construct
  REGION 1..13: note = Peptide Compound
  SITE 1: note = MISC_FEATURE - Xaa = BdpF
  SITE 3: note = MISC_FEATURE - Xaa = MeF
  SITE 6: note = MISC_FEATURE - Xaa = MeF
  SITE 9: note = MISC_FEATURE - Xaa = D-Ser(Ph)
  SITE 10: note = MISC_FEATURE - Xaa = MeA
XIXIGXIIXXIPG

SEQ ID NO: 17 - protein, 13 aa, synthetic construct
  REGION 1..13: note = Peptide Compound
  SITE 1: note = MISC_FEATURE - Xaa = BdpF
  SITE 3: note = MISC_FEATURE - Xaa = MeF
  SITE 6: note = MISC_FEATURE - Xaa = MeF
  SITE 9: note = MISC_FEATURE - Xaa = D-MeAbu
  SITE 10: note = MISC_FEATURE - Xaa = MeA
XIXIGXIIXXIPG

SEQ ID NO: 18 - protein, 13 aa, synthetic construct
  REGION 1..13: note = Peptide Compound
  SITE 1: note = MISC_FEATURE - Xaa = BdpF
  SITE 3: note = MISC_FEATURE - Xaa = MeF
  SITE 6: note = MISC_FEATURE - Xaa = MeF
  SITE 9: note = MISC_FEATURE - Xaa = D-MeSer
  SITE 10: note = MISC_FEATURE - Xaa = MeA
XIXIGXIIXXIPG

SEQ ID NO: 19 - protein, 13 aa, synthetic construct
  REGION 1..13: note = Peptide Compound
  SITE 1: note = MISC_FEATURE - Xaa = BdpF
  SITE 3: note = MISC_FEATURE - Xaa = MeF
  SITE 6: note = MISC_FEATURE - Xaa = MeF
  SITE 9: note = MISC_FEATURE - Xaa = D-Pro(4R-Bn)
  SITE 10: note = MISC_FEATURE - Xaa = MeA
XIXIGXIIXXIPG

SEQ ID NO: 20 - protein, 13 aa, synthetic construct
  REGION 1..13: note = Peptide Compound
  SITE 1: note = MISC_FEATURE - Xaa = BdpF
  SITE 3: note = MISC_FEATURE - Xaa = MeF
  SITE 6: note = MISC_FEATURE - Xaa = MeF
  SITE 9: note = MISC_FEATURE - Xaa = Hyp(Ph)
  SITE 10: note = MISC_FEATURE - Xaa = MeA
XIXIGXIIXXIPG

SEQ ID NO: 21 - protein, 13 aa, synthetic construct
  REGION 1..13: note = Peptide Compound
  SITE 1: note = MISC_FEATURE - Xaa = BdpF
  SITE 3: note = MISC_FEATURE - Xaa = MeF
  SITE 6: note = MISC_FEATURE - Xaa = MeF
  SITE 9: note = MISC_FEATURE - Xaa = nBuG
  SITE 10: note = MISC_FEATURE - Xaa = MeF
XIXIGXIIXXIPG

SEQ ID NO: 22 - protein, 13 aa, synthetic construct
  REGION 1..13: note = Peptide Compound
  SITE 1: note = MISC_FEATURE - Xaa = BdpF
  SITE 3: note = MISC_FEATURE - Xaa = MeF
  SITE 6: note = MISC_FEATURE - Xaa = MeF
  SITE 9: note = MISC_FEATURE - Xaa = MeOEtG
  SITE 10: note = MISC_FEATURE - Xaa = MeF
XIXIGXIIXXIPG

SEQ ID NO: 23 - protein, 13 aa, synthetic construct
  REGION 1..13: note = Peptide Compound
  SITE 1: note = MISC_FEATURE - Xaa = BdpF
  SITE 3: note = MISC_FEATURE - Xaa = MeF
  SITE 6: note = MISC_FEATURE - Xaa = MeF
  SITE 9: note = MISC_FEATURE - Xaa = MeOPrG
  SITE 10: note = MISC_FEATURE - Xaa = MeF
XIXIGXIIXXIPG

SEQ ID NO: 24 - protein, 13 aa, synthetic construct
  REGION 1..13: note = Peptide Compound
  SITE 1: note = MISC_FEATURE - Xaa = BdpF
  SITE 3: note = MISC_FEATURE - Xaa = MeF
  SITE 6: note = MISC_FEATURE - Xaa = MeF
  SITE 9: note = MISC_FEATURE - Xaa = PhPrG
  SITE 10: note = MISC_FEATURE - Xaa = MeF
XIXIGXIIXXIPG

SEQ ID NO: 25 - protein, 13 aa, synthetic construct
  REGION 1..13: note = Peptide Compound
  SITE 1: note = MISC_FEATURE - Xaa = BdpF
  SITE 3: note = MISC_FEATURE - Xaa = MeF
  SITE 6: note = MISC_FEATURE - Xaa = MeF
  SITE 9: note = MISC_FEATURE - Xaa = PhOEtG
  SITE 10: note = MISC_FEATURE - Xaa = MeF
XIXIGXIIXXIPG

SEQ ID NO: 26 - protein, 13 aa, synthetic construct
  REGION 1..13: note = Peptide Compound
  SITE 1: note = MISC_FEATURE - Xaa = BdpF
  SITE 3: note = MISC_FEATURE - Xaa = MeF
  SITE 6: note = MISC_FEATURE - Xaa = MeF
  SITE 9: note = MISC_FEATURE - Xaa = D-Nva
  SITE 10: note = MISC_FEATURE - Xaa = MeF
XIXIGXIIXXIPG

SEQ ID NO: 27 - protein, 13 aa, synthetic construct
  REGION 1..13: note = Peptide Compound
  SITE 1: note = MISC_FEATURE - Xaa = BdpF
  SITE 3: note = MISC_FEATURE - Xaa = MeF
  SITE 6: note = MISC_FEATURE - Xaa = MeF
  SITE 9: note = MISC_FEATURE - Xaa = D-Ser(Me)
  SITE 10: note = MISC_FEATURE - Xaa = MeF
XIXIGXIIXXIPG

SEQ ID NO: 28 - protein, 13 aa, synthetic construct
  REGION 1..13: note = Peptide Compound
  SITE 1: note = MISC_FEATURE - Xaa = BdpF
  SITE 3: note = MISC_FEATURE - Xaa = MeF
  SITE 6: note = MISC_FEATURE - Xaa = MeF
  SITE 9: note = MISC_FEATURE - Xaa = D-Hph
  SITE 10: note = MISC_FEATURE - Xaa = MeF
XIXIGXIIXXIPG

SEQ ID NO: 29 - protein, 13 aa, synthetic construct
  REGION 1..13: note = Peptide Compound
  SITE 1: note = MISC_FEATURE - Xaa = BdpF
  SITE 3: note = MISC_FEATURE - Xaa = MeF
  SITE 6: note = MISC_FEATURE - Xaa = MeF
  SITE 9: note = MISC_FEATURE - Xaa = D-Ser(Ph)
  SITE 10: note = MISC_FEATURE - Xaa = MeF
XIXIGXIIXXIPG

SEQ ID NO: 30 - protein, 13 aa, synthetic construct
  REGION 1..13: note = Peptide Compound
  SITE 1: note = MISC_FEATURE - Xaa = BdpF
  SITE 3: note = MISC_FEATURE - Xaa = MeF
  SITE 6: note = MISC_FEATURE - Xaa = MeF
  SITE 9: note = MISC_FEATURE - Xaa = D-MeAbu
  SITE 10: note = MISC_FEATURE - Xaa = MeF
XIXIGXIIXXIPG

SEQ ID NO: 31 - protein, 13 aa, synthetic construct
  REGION 1..13: note = Peptide Compound
  SITE 1: note = MISC_FEATURE - Xaa = BdpF
  SITE 3: note = MISC_FEATURE - Xaa = MeF
  SITE 6: note = MISC_FEATURE - Xaa = MeF
  SITE 9: note = MISC_FEATURE - Xaa = D-MeSer
  SITE 10: note = MISC_FEATURE - Xaa = MeF
XIXIGXIIXXIPG

SEQ ID NO: 32 - protein, 13 aa, synthetic construct
  REGION 1..13: note = Peptide Compound
  SITE 1: note = MISC_FEATURE - Xaa = BdpF
  SITE 3: note = MISC_FEATURE - Xaa = MeF
  SITE 6: note = MISC_FEATURE - Xaa = MeF
  SITE 9: note = MISC_FEATURE - Xaa = D-Pro(4R-Bn)
  SITE 10: note = MISC_FEATURE - Xaa = MeF
XIXIGXIIXXIPG

SEQ ID NO: 33 - protein, 13 aa, synthetic construct
  REGION 1..13: note = Peptide Compound
  SITE 1: note = MISC_FEATURE - Xaa = BdpF
  SITE 3: note = MISC_FEATURE - Xaa = MeF
  SITE 6: note = MISC_FEATURE - Xaa = MeF
  SITE 9: note = MISC_FEATURE - Xaa = Hyp(Ph)
  SITE 10: note = MISC_FEATURE - Xaa = MeF
XIXIGXIIXXIPG

SEQ ID NO: 34 - protein, 13 aa, synthetic construct
  REGION 1..13: note = Peptide Compound
  SITE 1: note = MISC_FEATURE - Xaa = BdpF
  SITE 3: note = MISC_FEATURE - Xaa = MeF
  SITE 6: note = MISC_FEATURE - Xaa = MeF
  SITE 9: note = MISC_FEATURE - Xaa = MeA
  SITE 10: note = MISC_FEATURE - Xaa = PhPrG
XIXIGXIIXXIPG

SEQ ID NO: 35 - protein, 13 aa, synthetic construct
  REGION 1..13: note = Peptide Compound
  SITE 1: note = MISC_FEATURE - Xaa = BdpF
  SITE 3: note = MISC_FEATURE - Xaa = MeF
  SITE 6: note = MISC_FEATURE - Xaa = MeF
  SITE 9: note = MISC_FEATURE - Xaa = MeA
  SITE 10: note = MISC_FEATURE - Xaa = PhOEtG
XIXIGXIIXXIPG

SEQ ID NO: 36 - protein, 13 aa, synthetic construct
  REGION 1..13: note = Peptide Compound
  SITE 1: note = MISC_FEATURE - Xaa = BdpF
  SITE 3: note = MISC_FEATURE - Xaa = MeF
  SITE 6: note = MISC_FEATURE - Xaa = MeF
  SITE 9: note = MISC_FEATURE - Xaa = MeF
  SITE 10: note = MISC_FEATURE - Xaa = PhPrG
XIXIGXIIXXIPG

SEQ ID NO: 37 - protein, 13 aa, synthetic construct
  REGION 1..13: note = Peptide Compound
  SITE 1: note = MISC_FEATURE - Xaa = BdpF
  SITE 3: note = MISC_FEATURE - Xaa = MeF
  SITE 6: note = MISC_FEATURE - Xaa = MeF
  SITE 9: note = MISC_FEATURE - Xaa = MeF
  SITE 10: note = MISC_FEATURE - Xaa = PhOEtG
XIXIGXIIXXIPG